European Patent Specification EP 3 775 902 B1, published February 22, 2023. Title: Diagnostic assays to detect tumor antigens in cancer patients. Applicant: F. Hoffmann-La Roche Ltd. The sequence listing filed with the application follows.

SEQUENCE LISTING (132 sequences)

SEQ ID NO: 1 - protein, 5 aa, Artificial sequence
  Anti-P329G CDR H1 Kabat
RYWMN

SEQ ID NO: 2 - protein, 17 aa, Artificial sequence
  Anti-P329G CDR H2
EITPDSSTINYTPSLKD

SEQ ID NO: 3 - protein, 10 aa, Artificial sequence
  Anti-P329G CDR H3 Kabat
PYDYGAWFAS

SEQ ID NO: 4 - protein, 14 aa, Artificial sequence
  Anti-P329G CDR L1 Kabat
RSSTGAVTTSNYAN

SEQ ID NO: 5 - protein, 7 aa, Artificial sequence
  Anti-P329G CDR L2 Kabat
GTNKRAP

SEQ ID NO: 6 - protein, 9 aa, Artificial sequence
  Anti-P329G CDR L3 Kabat
ALWYSNHWV

SEQ ID NO: 7 - protein, 433 aa, Artificial sequence
  Anti-P329G-ds-scFv-CD28ATD-CD28CSD-CD3zSSD fusion
EVKLLESGGGLVQPGGSLKLSCAASGFDFSRYWMNWVRQAPGKCLEWIGEITPDSSTINYTPSLKDKFIISRDNAKNTLYLQMIKVRSEDTALYYCVRPYDYGAWFASWGQGTLVTVSAGGGGSGGGGSGGGGSGGGGSQAVVTQESALTTSPGETVTLTCRSSTGAVTTSNYANWVQEKPDHLFTGLIGGTNKRAPGVPARFSGSLIGDKAALTITGAQTEDEAIYFCALWYSNHWVFGCGTKLTVLGGGGSFWVLVVVGGVLACYSLLVTVAFIIFWVRSKRSRLLHSDYMNMTPRRPGPTRKHYQPYAPPRDFAAYRSRVKFSRSADAPAYQQGQNQLYNELNLGRREEYDVLDKRRGRDPEMGGKPRRKNPQEGLYNELQKDKMAEAYSEIGMKGERRRGKGHDGLYQGLSTATKDTYDALHMQALPPR

SEQ ID NO: 8 - protein, 119 aa, Artificial sequence
  Anti-P329G-ds VH
EVKLLESGGGLVQPGGSLKLSCAASGFDFSRYWMNWVRQAPGKCLEWIGEITPDSSTINYTPSLKDKFIISRDNAKNTLYLQMIKVRSEDTALYYCVRPYDYGAWFASWGQGTLVTVSA

SEQ ID NO: 9 - protein, 109 aa, Artificial sequence
  Anti-P329G-ds VL
QAVVTQESALTTSPGETVTLTCRSSTGAVTTSNYANWVQEKPDHLFTGLIGGTNKRAPGVPARFSGSLIGDKAALTITGAQTEDEAIYFCALWYSNHWVFGCGTKLTVL

SEQ ID NO: 10 - protein, 248 aa, Artificial sequence
  Anti-P329G-ds-scFv
EVKLLESGGGLVQPGGSLKLSCAASGFDFSRYWMNWVRQAPGKCLEWIGEITPDSSTINYTPSLKDKFIISRDNAKNTLYLQMIKVRSEDTALYYCVRPYDYGAWFASWGQGTLVTVSAGGGGSGGGGSGGGGSGGGGSQAVVTQESALTTSPGETVTLTCRSSTGAVTTSNYANWVQEKPDHLFTGLIGGTNKRAPGVPARFSGSLIGDKAALTITGAQTEDEAIYFCALWYSNHWVFGCGTKLTVL

SEQ ID NO: 11 - protein, 27 aa, Artificial sequence
  CD28ATD
FWVLVVVGGVLACYSLLVTVAFIIFWV

SEQ ID NO: 12 - protein, 41 aa, Artificial sequence
  CD28CSD
RSKRSRLLHSDYMNMTPRRPGPTRKHYQPYAPPRDFAAYRS

SEQ ID NO: 13 - protein, 112 aa, Artificial sequence
  CD3zSSD
RVKFSRSADAPAYQQGQNQLYNELNLGRREEYDVLDKRRGRDPEMGGKPRRKNPQEGLYNELQKDKMAEAYSEIGMKGERRRGKGHDGLYQGLSTATKDTYDALHMQALPPR

SEQ ID NO: 14 - protein, 180 aa, Artificial sequence
  CD28ATD-CD28CSD-CD3zSSD
FWVLVVVGGVLACYSLLVTVAFIIFWVRSKRSRLLHSDYMNMTPRRPGPTRKHYQPYAPPRDFAAYRSRVKFSRSADAPAYQQGQNQLYNELNLGRREEYDVLDKRRGRDPEMGGKPRRKNPQEGLYNELQKDKMAEAYSEIGMKGERRRGKGHDGLYQGLSTATKDTYDALHMQALPPR

SEQ ID NO: 15 - protein, 238 aa, Artificial sequence
  eGFP
VSKGEELFTGVVPILVELDGDVNGHKFSVSGEGEGDATYGKLTLKFICTTGKLPVPWPTLVTTLTYGVQCFSRYPDHMKQHDFFKSAMPEGYVQERTIFFKDDGNYKTRAEVKFEGDTLVNRIELKGIDFKEDGNILGHKLEYNYNSHNVYIMADKQKNGIKVNFKIRHNIEDGSVQLADHYQQNTPIGDGPVLLPDNHYLSTQSALSKDPNEKRDHMVLLEFVTAAGITLGMDELYK

SEQ ID NO: 16 - protein, 20 aa, Artificial sequence
  (G4S)4 linker
GGGGSGGGGSGGGGSGGGGS

SEQ ID NO: 17 - protein, 5 aa, Artificial sequence
  G4S linker
GGGGS

SEQ ID NO: 18 - protein, 19 aa, Artificial sequence
  T2A linker
GEGRGSLLTCGDVEENPGP

SEQ ID NO: 19 - DNA, 1356 bp, Artificial sequence
  Anti-P329G-ds-scFv-CD28ATD-CD28CSD-CD3zSSD fusion
atgggatggagctgtatcatcctcttcttggtagcaacagctaccggtgtgcattccgaggtgaagctgctggagagcggcggcggcctggtgcagcccggcggcagcctgaagctgagctgcgccgccagcggcttcgacttcagcaggtactggatgaactgggtgaggcaggcccccggcaagtgtctggagtggatcggcgagatcacccccgacagcagcaccatcaactacacccccagcctgaaggacaagttcatcatcagcagggacaacgccaagaacaccctgtacctgcagatgatcaaggtgaggagcgaggacaccgccctgtactactgcgtgaggccctacgactacggcgcctggttcgccagctggggccagggcaccctggtgaccgtgagcgccggagggggcggaagtggtggcgggggaagcggcgggggtggcagcggagggggcggatctcaggccgtggtgacccaggagagcgccctgaccaccagccccggcgagaccgtgaccctgacctgcaggagcagcaccggcgccgtgaccaccagcaactacgccaactgggtgcaggagaagcccgaccacctgttcaccggcctgatcggcggcaccaacaagagggcccccggcgtgcccgccaggttcagcggcagcctgatcggcgacaaggccgccctgaccatcaccggcgcccagaccgaggacgaggccatctacttctgcgccctgtggtacagcaaccactgggtgttcggctgtggcaccaagctgaccgtgctgggagggggcggatccttctgggtgctggtggtggtgggcggcgtgctggcctgctacagcctgctggtgaccgtggccttcatcatcttctgggtgaggagcaagaggagcaggctgctgcacagcgactacatgaacatgacccccaggaggcccggccccaccaggaagcactaccagccctacgccccccccagggacttcgccgcctacaggagcagggtgaagttcagcaggagcgccgacgcccccgcctaccagcagggccagaaccagctgtataacgagctgaacctgggcaggagggaggagtacgacgtgctggacaagaggaggggcagggaccccgagatgggcggcaagcccaggaggaagaacccccaggagggcctgtataacgagctgcagaaggacaagatggccgaggcctacagcgagatcggcatgaagggcgagaggaggaggggcaagggccacgacggcctgtaccagggcctgagcaccgccaccaaggacacctacgacgccctgcacatgcaggccctgccccccagg

SEQ ID NO: 20 - DNA, 357 bp, Artificial sequence
  Anti-P329G-ds VH
gaggtgaagctgctggagagcggcggcggcctggtgcagcccggcggcagcctgaagctgagctgcgccgccagcggcttcgacttcagcaggtactggatgaactgggtgaggcaggcccccggcaagtgtctggagtggatcggcgagatcacccccgacagcagcaccatcaactacacccccagcctgaaggacaagttcatcatcagcagggacaacgccaagaacaccctgtacctgcagatgatcaaggtgaggagcgaggacaccgccctgtactactgcgtgaggccctacgactacggcgcctggttcgccagctggggccagggcaccctggtgaccgtgagcgcc

SEQ ID NO: 21 - DNA, 327 bp, Artificial sequence
  Anti-P329G-ds VL
caggccgtggtgacccaggagagcgccctgaccaccagccccggcgagaccgtgaccctgacctgcaggagcagcaccggcgccgtgaccaccagcaactacgccaactgggtgcaggagaagcccgaccacctgttcaccggcctgatcggcggcaccaacaagagggcccccggcgtgcccgccaggttcagcggcagcctgatcggcgacaaggccgccctgaccatcaccggcgcccagaccgaggacgaggccatctacttctgcgccctgtggtacagcaaccactgggtgttcggctgtggcaccaagctgaccgtgctg

SEQ ID NO: 22 - DNA, 801 bp, Artificial sequence
  Anti-P329G-ds-scFv
atgggatggagctgtatcatcctcttcttggtagcaacagctaccggtgtgcattccgaggtgaagctgctggagagcggcggcggcctggtgcagcccggcggcagcctgaagctgagctgcgccgccagcggcttcgacttcagcaggtactggatgaactgggtgaggcaggcccccggcaagtgtctggagtggatcggcgagatcacccccgacagcagcaccatcaactacacccccagcctgaaggacaagttcatcatcagcagggacaacgccaagaacaccctgtacctgcagatgatcaaggtgaggagcgaggacaccgccctgtactactgcgtgaggccctacgactacggcgcctggttcgccagctggggccagggcaccctggtgaccgtgagcgccggagggggcggaagtggtggcgggggaagcggcgggggtggcagcggagggggcggatctcaggccgtggtgacccaggagagcgccctgaccaccagccccggcgagaccgtgaccctgacctgcaggagcagcaccggcgccgtgaccaccagcaactacgccaactgggtgcaggagaagcccgaccacctgttcaccggcctgatcggcggcaccaacaagagggcccccggcgtgcccgccaggttcagcggcagcctgatcggcgacaaggccgccctgaccatcaccggcgcccagaccgaggacgaggccatctacttctgcgccctgtggtacagcaaccactgggtgttcggctgtggcaccaagctgaccgtgctg

SEQ ID NO: 23 - DNA, 81 bp, Artificial sequence
  CD28ATD
ttctgggtgctggtggtggtgggcggcgtgctggcctgctacagcctgctggtgaccgtggccttcatcatcttctgggtg

SEQ ID NO: 24 - DNA, 123 bp, Artificial sequence
  CD28CSD
aggagcaagaggagcaggctgctgcacagcgactacatgaacatgacccccaggaggcccggccccaccaggaagcactaccagccctacgccccccccagggacttcgccgcctacaggagc

SEQ ID NO: 25 - DNA, 336 bp, Artificial sequence
  CD3zSSD
agggtgaagttcagcaggagcgccgacgcccccgcctaccagcagggccagaaccagctgtataacgagctgaacctgggcaggagggaggagtacgacgtgctggacaagaggaggggcagggaccccgagatgggcggcaagcccaggaggaagaacccccaggagggcctgtataacgagctgcagaaggacaagatggccgaggcctacagcgagatcggcatgaagggcgagaggaggaggggcaagggccacgacggcctgtaccagggcctgagcaccgccaccaaggacacctacgacgccctgcacatgcaggccctgccccccagg

SEQ ID NO: 26 - DNA, 540 bp, Artificial sequence
  CD28ATD-CD28CSD-CD3zSSD
ttctgggtgctggtggtggtgggcggcgtgctggcctgctacagcctgctggtgaccgtggccttcatcatcttctgggtgaggagcaagaggagcaggctgctgcacagcgactacatgaacatgacccccaggaggcccggccccaccaggaagcactaccagccctacgccccccccagggacttcgccgcctacaggagcagggtgaagttcagcaggagcgccgacgcccccgcctaccagcagggccagaaccagctgtataacgagctgaacctgggcaggagggaggagtacgacgtgctggacaagaggaggggcagggaccccgagatgggcggcaagcccaggaggaagaacccccaggagggcctgtataacgagctgcagaaggacaagatggccgaggcctacagcgagatcggcatgaagggcgagaggaggaggggcaagggccacgacggcctgtaccagggcctgagcaccgccaccaaggacacctacgacgccctgcacatgcaggccctgccccccagg

SEQ ID NO: 27 - DNA, 63 bp, Artificial sequence
  T2A element
tccggagagggcagaggaagtcttctaacatgcggtgacgtggaggagaatcccggccctagg

SEQ ID NO: 28 - DNA, 717 bp, Artificial sequence
  eGFP
gtgagcaagggcgaggagctgttcaccggggtggtgcccatcctggtcgagctggacggcgacgtaaacggccacaagttcagcgtgtccggcgagggcgagggcgatgccacctacggcaagctgaccctgaagttcatctgcaccaccggcaagctgcccgtgccctggcccaccctcgtgaccaccctgacctacggcgtgcagtgcttcagccgctaccccgaccacatgaagcagcacgacttcttcaagtccgccatgcccgaaggctacgtccaggagcgcaccatcttcttcaaggacgacggcaactacaagacccgcgccgaggtgaagttcgagggcgacaccctggtgaaccgcatcgagctgaagggcatcgacttcaaggaggacggcaacatcctggggcacaagctggagtacaactacaacagccacaacgtctatatcatggccgacaagcagaagaacggcatcaaggtgaacttcaagatccgccacaacatcgaggacggcagcgtgcagctcgccgaccactaccagcagaacacccccatcggcgacggccccgtgctgctgcccgacaaccactacctgagcacccagtccgccctgagcaaagaccccaacgagaagcgcgatcacatggtcctgctggagttcgtgaccgccgccgggatcactctcggcatggacgagctgtacaagtga

SEQ ID NO: 29 - DNA, 2136 bp, Artificial sequence
  Anti-P329G-ds-scFv-CD28ATD-CD28CSD-CD3zSSD-eGFP fusion
atgggatggagctgtatcatcctcttcttggtagcaacagctaccggtgtgcattccgaggtgaagctgctggagagcggcggcggcctggtgcagcccggcggcagcctgaagctgagctgcgccgccagcggcttcgacttcagcaggtactggatgaactgggtgaggcaggcccccggcaagtgtctggagtggatcggcgagatcacccccgacagcagcaccatcaactacacccccagcctgaaggacaagttcatcatcagcagggacaacgccaagaacaccctgtacctgcagatgatcaaggtgaggagcgaggacaccgccctgtactactgcgtgaggccctacgactacggcgcctggttcgccagctggggccagggcaccctggtgaccgtgagcgccggagggggcggaagtggtggcgggggaagcggcgggggtggcagcggagggggcggatctcaggccgtggtgacccaggagagcgccctgaccaccagccccggcgagaccgtgaccctgacctgcaggagcagcaccggcgccgtgaccaccagcaactacgccaactgggtgcaggagaagcccgaccacctgttcaccggcctgatcggcggcaccaacaagagggcccccggcgtgcccgccaggttcagcggcagcctgatcggcgacaaggccgccctgaccatcaccggcgcccagaccgaggacgaggccatctacttctgcgccctgtggtacagcaaccactgggtgttcggctgtggcaccaagctgaccgtgctgggagggggcggatccttctgggtgctggtggtggtgggcggcgtgctggcctgctacagcctgctggtgaccgtggccttcatcatcttctgggtgaggagcaagaggagcaggctgctgcacagcgactacatgaacatgacccccaggaggcccggccccaccaggaagcactaccagccctacgccccccccagggacttcgccgcctacaggagcagggtgaagttcagcaggagcgccgacgcccccgcctaccagcagggccagaaccagctgtataacgagctgaacctgggcaggagggaggagtacgacgtgctggacaagaggaggggcagggaccccgagatgggcggcaagcccaggaggaagaacccccaggagggcctgtataacgagctgcagaaggacaagatggccgaggcctacagcgagatcggcatgaagggcgagaggaggaggggcaagggccacgacggcctgtaccagggcctgagcaccgccaccaaggacacctacgacgccctgcacatgcaggccctgccccccaggtccggagagggcagaggaagtcttctaacatgcggtgacgtggaggagaatcccggccctagggtgagcaagggcgaggagctgttcaccggggtggtgcccatcctggtcgagctggacggcgacgtaaacggccacaagttcagcgtgtccggcgagggcgagggcgatgccacctacggcaagctgaccctgaagttcatctgcaccaccggcaagctgcccgtgccctggcccaccctcgtgaccaccctgacctacggcgtgcagtgcttcagccgctaccccgaccacatgaagcagcacgacttcttcaagtccgccatgcccgaaggctacgtccaggagcgcaccatcttcttcaaggacgacggcaactacaagacccgcgccgaggtgaagttcgagggcgacaccctggtgaaccgcatcgagctgaagggcatcgacttcaaggaggacggcaacatcctggggcacaagctggagtacaactacaacagccacaacgtctatatcatggccgacaagcagaagaacggcatcaaggtgaacttcaagatccgccacaacatcgaggacggcagcgtgcagctcgccgaccactaccagcagaacacccccatcggcgacggccccgtgctgctgcccgacaaccactacctgagcacccagtccgccctgagcaaagaccccaacgagaagcgcgatcacatggtcctgctggagttcgtgaccgccgccgggatcactctcggcatggacgagctgtacaagtga

SEQ ID NO: 30 - protein, 407 aa, Artificial sequence
  Anti-P329G-Fab-heavy chain- CD28ATD-CD28CSD-CD3zSSD fusion
EVKLLESGGGLVQPGGSLKLSCAASGFDFSRYWMNWVRQAPGKGLEWIGEITPDSSTINYTPSLKDKFIISRDNAKNTLYLQMIKVRSEDTALYYCVRPYDYGAWFASWGQGTLVTVSAASTKGPSVFPLAPSSKSTSGGTAALGCLVKDYFPEPVTVSWNSGALTSGVHTFPAVLQSSGLYSLSSVVTVPSSSLGTQTYICNVNHKPSNTKVDKKVEPKSCGGGGSFWVLVVVGGVLACYSLLVTVAFIIFWVRSKRSRLLHSDYMNMTPRRPGPTRKHYQPYAPPRDFAAYRSRVKFSRSADAPAYQQGQNQLYNELNLGRREEYDVLDKRRGRDPEMGGKPRRKNPQEGLYNELQKDKMAEAYSEIGMKGERRRGKGHDGLYQGLSTATKDTYDALHMQALPPR

SEQ ID NO: 31 - protein, 222 aa, Artificial sequence
  Anti-P329G-Fab heavy chain
EVKLLESGGGLVQPGGSLKLSCAASGFDFSRYWMNWVRQAPGKGLEWIGEITPDSSTINYTPSLKDKFIISRDNAKNTLYLQMIKVRSEDTALYYCVRPYDYGAWFASWGQGTLVTVSAASTKGPSVFPLAPSSKSTSGGTAALGCLVKDYFPEPVTVSWNSGALTSGVHTFPAVLQSSGLYSLSSVVTVPSSSLGTQTYICNVNHKPSNTKVDKKVEPKSC

SEQ ID NO: 32 - protein, 216 aa, Artificial sequence
  Anti-P329G-Fab light chain
QAVVTQESALTTSPGETVTLTCRSSTGAVTTSNYANWVQEKPDHLFTGLIGGTNKRAPGVPARFSGSLIGDKAALTITGAQTEDEAIYFCALWYSNHWVFGGGTKLTVLRTVAAPSVFIFPPSDEQLKSGTASVVCLLNNFYPREAKVQWKVDNALQSGNSQESVTEQDSKDSTYSLSSTLTLSKADYEKHKVYACEVTHQGLSSPVTKSFNRGEC

SEQ ID NO: 33 - protein, 109 aa, Artificial sequence
  Anti-P329G VL
QAVVTQESALTTSPGETVTLTCRSSTGAVTTSNYANWVQEKPDHLFTGLIGGTNKRAPGVPARFSGSLIGDKAALTITGAQTEDEAIYFCALWYSNHWVFGGGTKLTVL

SEQ ID NO: 34 - protein, 107 aa, Artificial sequence [sequence omitted]

SEQ ID NO: 35 - protein, 119 aa, Artificial sequence
  Anti-P329G VH
EVKLLESGGGLVQPGGSLKLSCAASGFDFSRYWMNWVRQAPGKGLEWIGEITPDSSTINYTPSLKDKFIISRDNAKNTLYLQMIKVRSEDTALYYCVRPYDYGAWFASWGQGTLVTVSA

SEQ ID NO: 36 - protein, 103 aa, Artificial sequence
  CH1
ASTKGPSVFPLAPSSKSTSGGTAALGCLVKDYFPEPVTVSWNSGALTSGVHTFPAVLQSSGLYSLSSVVTVPSSSLGTQTYICNVNHKPSNTKVDKKVEPKSC

SEQ ID NO: 37 - DNA, 2645 bp, Artificial sequence
  Anti-P329G-Fab-heavy chain- CD28ATD-CD28CSD-CD3zSSD fusion
atgggatggagctgtatcatcctcttcttggtagcaacagctacgggtgtgcattcccaggccgtggtgacccaggagagcgccctgaccaccagccccggcgagaccgtgaccctgacctgcaggagcagcaccggcgccgtgaccaccagcaactacgccaactgggtgcaggagaagcccgaccacctgttcaccggcctgatcggcggcaccaacaagagggcccccggcgtgcccgccaggttcagcggcagcctgatcggcgacaaggccgccctgaccatcaccggcgcccagaccgaggacgaggccatctacttctgcgccctgtggtacagcaaccactgggtgttcggcggtggcaccaagctgaccgtgctgcgtacggtggctgcaccatctgtcttcatcttcccgccatctgatgagcagttgaaatctggaactgcctctgttgtgtgcctgctgaataacttctatcccagagaggccaaagtacagtggaaggtggataacgccctccaatcgggtaactcccaggagagtgtcacagagcaggacagcaaggacagcacctacagcctcagcagcaccctgacgctgagcaaagcagactacgagaaacacaaagtctacgcctgcgaagtcacccatcagggcctgagctcgcccgtcacaaagagcttcaacaggggagagtgttaggaattccccgaagtaacttagaagctgtaaatcaacgatcaatagcaggtgtggcacaccagtcataccttgatcaagcacttctgtttccccggactgagtatcaataggctgctcgcgcggctgaaggagaaaacgttcgttacccgaccaactacttcgagaagcttagtaccaccatgaacgaggcagggtgtttcgctcagcacaaccccagtgtagatcaggctgatgagtcactgcaacccccatgggcgaccatggcagtggctgcgttggcggcctgcccatggagaaatccatgggacgctctaattctgacatggtgtgaagtgcctattgagctaactggtagtcctccggcccctgattgcggctaatcctaactgcggagcacatgctcacaaaccagtgggtggtgtgtcgtaacgggcaactctgcagcggaaccgactactttgggtgtccgtgtttccttttattcctatattggctgcttatggtgacaatcaaaaagttgttaccatatagctattggattggccatccggtgtgcaacagggcaactgtttacctatttattggttttgtaccattatcactgaagtctgtgatcactctcaaattcattttgaccctcaacacaatcaaacgccaccatgggatggagctgtatcatcctcttcttggtagcaacagctaccggtgtgcactccgaggtgaagctgctggagagcggcggcggcctggtgcagcccggcggcagcctgaagctgagctgcgccgccagcggcttcgacttcagcaggtactggatgaactgggtgaggcaggcccccggcaagggtctggagtggatcggcgagatcacccccgacagcagcaccatcaactacacccccagcctgaaggacaagttcatcatcagcagggacaacgccaagaacaccctgtacctgcagatgatcaaggtgaggagcgaggacaccgccctgtactactgcgtgaggccctacgactacggcgcctggttcgccagctggggccagggcaccctggtgaccgtgagcgccgctagcaccaagggcccctccgtgttccccctggcccccagcagcaagagcaccagcggcggcacagccgctctgggctgcctggtcaaggactacttccccgagcccgtgaccgtgtcctggaacagcggagccctgacctccggcgtgcacaccttccccgccgtgctgcagagttctggcctgtatagcctgagcagcgtggtcaccgtgccttctagcagcctgggcacccagacctacatctgcaacgtgaaccacaagcccagcaacaccaaggtggacaagaaggtggagcccaagagctgcggagggggcggatccttctgggtgctggtggtggtgggcggcgtgctggcctgctacagcctgctggtgaccgtggccttcatcatcttctgggtgaggagcaagaggagcaggctgctgcacagcgactacatgaacatgacccccaggaggcccggccccaccaggaagcactaccagccctacgccccccccagggacttcgccgcctacaggagcagggtgaagttcagcaggagcgccgacgcccccgcctaccagcagggccagaaccagctgtataacgagctgaacctgggcaggagggaggagtacgacgtgctggacaagaggaggggcagggaccccgagatgggcggcaagcccaggaggaagaacccccaggagggcctgtataacgagctgcagaaggacaagatggccgaggcctacagcgagatcggcatgaagggcgagaggaggaggggcaagggccacgacggcctgtaccagggcctgagcaccgccaccaaggacacctacgacgccctgcacatgcaggccctgccccccagg

SEQ ID NO: 38 - DNA, 327 bp, Artificial sequence
  Anti-P329G VL
caggccgtggtgacccaggagagcgccctgaccaccagccccggcgagaccgtgaccctgacctgcaggagcagcaccggcgccgtgaccaccagcaactacgccaactgggtgcaggagaagcccgaccacctgttcaccggcctgatcggcggcaccaacaagagggcccccggcgtgcccgccaggttcagcggcagcctgatcggcgacaaggccgccctgaccatcaccggcgcccagaccgaggacgaggccatctacttctgcgccctgtggtacagcaaccactgggtgttcggcggtggcaccaagctgaccgtgctg

SEQ ID NO: 39 - DNA, 324 bp, Artificial sequence
  CL
cgtacggtggctgcaccatctgtcttcatcttcccgccatctgatgagcagttgaaatctggaactgcctctgttgtgtgcctgctgaataacttctatcccagagaggccaaagtacagtggaaggtggataacgccctccaatcgggtaactcccaggagagtgtcacagagcaggacagcaaggacagcacctacagcctcagcagcaccctgacgctgagcaaagcagactacgagaaacacaaagtctacgcctgcgaagtcacccatcagggcctgagctcgcccgtcacaaagagcttcaacaggggagagtgttag

SEQ ID NO: 40 - DNA, 357 bp, Artificial sequence
  Anti-P329G VH
gaggtgaagctgctggagagcggcggcggcctggtgcagcccggcggcagcctgaagctgagctgcgccgccagcggcttcgacttcagcaggtactggatgaactgggtgaggcaggcccccggcaagggtctggagtggatcggcgagatcacccccgacagcagcaccatcaactacacccccagcctgaaggacaagttcatcatcagcagggacaacgccaagaacaccctgtacctgcagatgatcaaggtgaggagcgaggacaccgccctgtactactgcgtgaggccctacgactacggcgcctggttcgccagctggggccagggcaccctggtgaccgtgagcgcc

SEQ ID NO: 41 - DNA, 309 bp, Artificial sequence
  CH1
gctagcaccaagggcccctccgtgttccccctggcccccagcagcaagagcaccagcggcggcacagccgctctgggctgcctggtcaaggactacttccccgagcccgtgaccgtgtcctggaacagcggagccctgacctccggcgtgcacaccttccccgccgtgctgcagagttctggcctgtatagcctgagcagcgtggtcaccgtgccttctagcagcctgggcacccagacctacatctgcaacgtgaaccacaagcccagcaacaccaaggtggacaagaaggtggagcccaagagctgc

SEQ ID NO: 42 - DNA, 647 bp, Artificial sequence
  IRES EV71, internal ribosomal entry side
cccgaagtaacttagaagctgtaaatcaacgatcaatagcaggtgtggcacaccagtcataccttgatcaagcacttctgtttccccggactgagtatcaataggctgctcgcgcggctgaaggagaaaacgttcgttacccgaccaactacttcgagaagcttagtaccaccatgaacgaggcagggtgtttcgctcagcacaaccccagtgtagatcaggctgatgagtcactgcaacccccatgggcgaccatggcagtggctgcgttggcggcctgcccatggagaaatccatgggacgctctaattctgacatggtgtgaagtgcctattgagctaactggtagtcctccggcccctgattgcggctaatcctaactgcggagcacatgctcacaaaccagtgggtggtgtgtcgtaacgggcaactctgcagcggaaccgactactttgggtgtccgtgtttccttttattcctatattggctgcttatggtgacaatcaaaaagttgttaccatatagctattggattggccatccggtgtgcaacagggcaactgtttacctatttattggttttgtaccattatcactgaagtctgtgatcactctcaaattcattttgaccctcaacacaatcaaac

SEQ ID NO: 43 - DNA, 3425 bp, Artificial sequence
  Anti-P329G-Fab-heavy chain- CD28ATD-CD28CSD-CD3zSSD-eGFP fusion
atgggatggagctgtatcatcctcttcttggtagcaacagctacgggtgtgcattcccaggccgtggtgacccaggagagcgccctgaccaccagccccggcgagaccgtgaccctgacctgcaggagcagcaccggcgccgtgaccaccagcaactacgccaactgggtgcaggagaagcccgaccacctgttcaccggcctgatcggcggcaccaacaagagggcccccggcgtgcccgccaggttcagcggcagcctgatcggcgacaaggccgccctgaccatcaccggcgcccagaccgaggacgaggccatctacttctgcgccctgtggtacagcaaccactgggtgttcggcggtggcaccaagctgaccgtgctgcgtacggtggctgcaccatctgtcttcatcttcccgccatctgatgagcagttgaaatctggaactgcctctgttgtgtgcctgctgaataacttctatcccagagaggccaaagtacagtggaaggtggataacgccctccaatcgggtaactcccaggagagtgtcacagagcaggacagcaaggacagcacctacagcctcagcagcaccctgacgctgagcaaagcagactacgagaaacacaaagtctacgcctgcgaagtcacccatcagggcctgagctcgcccgtcacaaagagcttcaacaggggagagtgttaggaattccccgaagtaacttagaagctgtaaatcaacgatcaatagcaggtgtggcacaccagtcataccttgatcaagcacttctgtttccccggactgagtatcaataggctgctcgcgcggctgaaggagaaaacgttcgttacccgaccaactacttcgagaagcttagtaccaccatgaacgaggcagggtgtttcgctcagcacaaccccagtgtagatcaggctgatgagtcactgcaacccccatgggcgaccatggcagtggctgcgttggcggcctgcccatggagaaatccatgggacgctctaattctgacatggtgtgaagtgcctattgagctaactggtagtcctccggcccctgattgcggctaatcctaactgcggagcacatgctcacaaaccagtgggtggtgtgtcgtaacgggcaactctgcagcggaaccgactactttgggtgtccgtgtttccttttattcctatattggctgcttatggtgacaatcaaaaagttgttaccatatagctattggattggccatccggtgtgcaacagggcaactgtttacctatttattggttttgtaccattatcactgaagtctgtgatcactctcaaattcattttgaccctcaacacaatcaaacgccaccatgggatggagctgtatcatcctcttcttggtagcaacagctaccggtgtgcactccgaggtgaagctgctggagagcggcggcggcctggtgcagcccggcggcagcctgaagctgagctgcgccgccagcggcttcgacttcagcaggtactggatgaactgggtgaggcaggcccccggcaagggtctggagtggatcggcgagatcacccccgacagcagcaccatcaactacacccccagcctgaaggacaagttcatcatcagcagggacaacgccaagaacaccctgtacctgcagatgatcaaggtgaggagcgaggacaccgccctgtactactgcgtgaggccctacgactacggcgcctggttcgccagctggggccagggcaccctggtgaccgtgagcgccgctagcaccaagggcccctccgtgttccccctggcccccagcagcaagagcaccagcggcggcacagccgctctgggctgcctggtcaaggactacttccccgagcccgtgaccgtgtcctggaacagcggagccctgacctccggcgtgcacaccttccccgccgtgctgcagagttctggcctgtatagcctgagcagcgtggtcaccgtgccttctagcagcctgggcacccagacctacatctgcaacgtgaaccacaagcccagcaacaccaaggtggacaagaaggtggagcccaagagctgcggagggggcggatccttctgggtgctggtggtggtgggcggcgtgctggcctgctacagcctgctggtgaccgtggccttcatcatcttctgggtgaggagcaagaggagcaggctgctgcacagcgactacatgaacatgacccccaggaggcccggccccaccaggaagcactaccagccctacgccccccccagggacttcgccgcctacaggagcagggtgaagttcagcaggagcgccgacgcccccgcctaccagcagggccagaaccagctgtataacgagctgaacctgggcaggagggaggagtacgacgtgctggacaagaggaggggcagggaccccgagatgggcggcaagcccaggaggaagaacccccaggagggcctgtataacgagctgcagaaggacaagatggccgaggcctacagcgagatcggcatgaagggcgagaggaggaggggcaagggccacgacggcctgtaccagggcctgagcaccgccaccaaggacacctacgacgccctgcacatgcaggccctgccccccaggtccggagagggcagaggaagtcttctaacatgcggtgacgtggaggagaatcccggccctagggtgagcaagggcgaggagctgttcaccggggtggtgcccatcctggtcgagctggacggcgacgtaaacggccacaagttcagcgtgtccggcgagggcgagggcgatgccacctacggcaagctgaccctgaagttcatctgcaccaccggcaagctgcccgtgccctggcccaccctcgtgaccaccctgacctacggcgtgcagtgcttcagccgctaccccgaccacatgaagcagcacgacttcttcaagtccgccatgcccgaaggctacgtccaggagcgcaccatcttcttcaaggacgacggcaactacaagacccgcgccgaggtgaagttcgagggcgacaccctggtgaaccgcatcgagctgaagggcatcgacttcaaggaggacggcaacatcctggggcacaagctggagtacaactacaacagccacaacgtctatatcatggccgacaagcagaagaacggcatcaaggtgaacttcaagatccgccacaacatcgaggacggcagcgtgcagctcgccgaccactaccagcagaacacccccatcggcgacggccccgtgctgctgcccgacaaccactacctgagcacccagtccgccctgagcaaagaccccaacgagaagcgcgatcacatggtcctgctggagttcgtgaccgccgccgggatcactctcggcatggacgagctgtacaagtga

SEQ ID NO: 44 - protein, 5 aa, Artificial sequence
  Anti-AAA CDR H1 Kabat
SYGMS

SEQ ID NO: 45 - protein, 6 aa, Artificial sequence
  Anti-AAA CDR H2 Kabat
SSGGSY

SEQ ID NO: 46 - protein, 12 aa, Artificial sequence
  Anti-AAA CDR H3 Kabat
LGMITTGYAMDY

SEQ ID NO: 47 - protein, 16 aa, Artificial sequence
  Anti-AAA CDR L1 Kabat
RSSQTIVHSTGHTYLE

SEQ ID NO: 48 - protein, 7 aa, Artificial sequence
  Anti-AAA CDR L2 Kabat
KVSNRFS

SEQ ID NO: 49 - protein, 9 aa, Artificial sequence
  Anti-AAA CDR L3 Kabat
FQGSHVPYT

SEQ ID NO: 50 - protein, 457 aa, Artificial sequence
  Anti-AAA-scFv-CD28ATD-CD28CSD-CD3zSSD fusion
MNFGLSLVFLALILKGVQCEVQLVESGGDLVKPGGSLKLSCAASGFTFSSYGMSWVRQTPDKRLEWVATISSGGSYIYYPDSVKGRFTISRDNAKNTLYLQMSSLKSEDTAMYYCARLGMITTGYAMDYWGQGTSVTVSSGGGGSGGGGSGGGGSGGGGSDVLMTQTPLSLPVSLGDQASISCRSSQTIVHSTGHTYLEWFLQKPGQSPKLLIYKVSNRFSGVPDRFSGSGSGTDFTLKISRVEAEDLGVYYCFQGSHVPYTFGGGTKLEIKGGGGSFWVLVVVGGVLACYSLLVTVAFIIFWVRSKRSRLLHSDYMNMTPRRPGPTRKHYQPYAPPRDFAAYRSRVKFSRSADAPAYQQGQNQLYNELNLGRREEYDVLDKRRGRDPEMGGKPRRKNPQEGLYNELQKDKMAEAYSEIGMKGERRRGKGHDGLYQGLSTATKDTYDALHMQALPPR

SEQ ID NO: 51 - protein, 272 aa, Artificial sequence
  Anti-AAA-scFv
MNFGLSLVFLALILKGVQCEVQLVESGGDLVKPGGSLKLSCAASGFTFSSYGMSWVRQTPDKRLEWVATISSGGSYIYYPDSVKGRFTISRDNAKNTLYLQMSSLKSEDTAMYYCARLGMITTGYAMDYWGQGTSVTVSSGGGGSGGGGSGGGGSGGGGSDVLMTQTPLSLPVSLGDQASISCRSSQTIVHSTGHTYLEWFLQKPGQSPKLLIYKVSNRFSGVPDRFSGSGSGTDFTLKISRVEAEDLGVYYCFQGSHVPYTFGGGTKLEIK

SEQ ID NO: 52 - protein, 140 aa, Artificial sequence
  Anti-AAA VH
MNFGLSLVFLALILKGVQCEVQLVESGGDLVKPGGSLKLSCAASGFTFSSYGMSWVRQTPDKRLEWVATISSGGSYIYYPDSVKGRFTISRDNAKNTLYLQMSSLKSEDTAMYYCARLGMITTGYAMDYWGQGTSVTVSS

SEQ ID NO: 53 - protein, 112 aa, Artificial sequence
  Anti-AAA VL
DVLMTQTPLSLPVSLGDQASISCRSSQTIVHSTGHTYLEWFLQKPGQSPKLLIYKVSNRFSGVPDRFSGSGSGTDFTLKISRVEAEDLGVYYCFQGSHVPYTFGGGTKLEIK

SEQ ID NO: 54 - protein, 428 aa, Artificial sequence
  Anti-AAA-Fab-heavy chain-CD28ATD-CD28CSD-CD3zSSD fusion
MNFGLSLVFLALILKGVQCEVQLVESGGDLVKPGGSLKLSCAASGFTFSSYGMSWVRQTPDKRLEWVATISSGGSYIYYPDSVKGRFTISRDNAKNTLYLQMSSLKSEDTAMYYCARLGMITTGYAMDYWGQGTSVTVSSASTKGPSVFPLAPSSKSTSGGTAALGCLVKDYFPEPVTVSWNSGALTSGVHTFPAVLQSSGLYSLSSVVTVPSSSLGTQTYICNVNHKPSNTKVDKKVEPKSCGGGGSFWVLVVVGGVLACYSLLVTVAFIIFWVRSKRSRLLHSDYMNMTPRRPGPTRKHYQPYAPPRDFAAYRSRVKFSRSADAPAYQQGQNQLYNELNLGRREEYDVLDKRRGRDPEMGGKPRRKNPQEGLYNELQKDKMAEAYSEIGMKGERRRGKGHDGLYQGLSTATKDTYDALHMQALPPR

SEQ ID NO: 55 - protein, 243 aa, Artificial sequence
  Anti-AAA-Fab heavy chain
MNFGLSLVFLALILKGVQCEVQLVESGGDLVKPGGSLKLSCAASGFTFSSYGMSWVRQTPDKRLEWVATISSGGSYIYYPDSVKGRFTISRDNAKNTLYLQMSSLKSEDTAMYYCARLGMITTGYAMDYWGQGTSVTVSSASTKGPSVFPLAPSSKSTSGGTAALGCLVKDYFPEPVTVSWNSGALTSGVHTFPAVLQSSGLYSLSSVVTVPSSSLGTQTYICNVNHKPSNTKVDKKVEPKSC

SEQ ID NO: 56 - protein, 219 aa, Artificial sequence
  Anti-AAA-Fab light chain
DVLMTQTPLSLPVSLGDQASISCRSSQTIVHSTGHTYLEWFLQKPGQSPKLLIYKVSNRFSGVPDRFSGSGSGTDFTLKISRVEAEDLGVYYCFQGSHVPYTFGGGTKLEIKRTVAAPSVFIFPPSDEQLKSGTASVVCLLNNFYPREAKVQWKVDNALQSGNSQESVTEQDSKDSTYSLSSTLTLSKADYEKHKVYACEVTHQGLSSPVTKSFNRGEC

SEQ ID NO: 57 - protein, 5 aa, Artificial sequence
  Anti-DIG CDR H1 Kabat
DYAMS

SEQ ID NO: 58 - protein, 17 aa, Artificial sequence
  Anti-DIG CDR H2 Kabat
SINIGATYIYYADSVKG

SEQ ID NO: 59 - protein, 16 aa, Artificial sequence
  Anti-DIG CDR H3 Kabat
PGSPYEYDKAYYSMAY

SEQ ID NO: 60 - protein, 11 aa, Artificial sequence
  Anti-DIG CDR L1 Kabat
RASQDIKNYLN

SEQ ID NO: 61 - protein, 7 aa, Artificial sequence
  Anti-DIG CDR L2 Kabat
YSSTLLS

SEQ ID NO: 62 - protein, 9 aa, Artificial sequence
  Anti-DIG CDR L3 Kabat
QQSITLPPT

SEQ ID NO: 63 - protein, 437 aa, Artificial sequence
  Anti-DIG-ds-scFv-CD28ATD-CD28CSD-CD3zSSD fusion
QVQLVESGGGLVKPGGSLRLSCAASGFTFSDYAMSWIRQAPGKCLEWVSSINIGATYIYYADSVKGRFTISRDNAKNSLYLQMNSLRAEDTAVYYCARPGSPYEYDKAYYSMAYWGQGTTVTVSSGGGGSGGGGSGGGGSGGGGSDIQMTQSPSSLSASVGDRVTITCRASQDIKNYLNWYQQKPGKAPKLLIYYSSTLLSGVPSRFSGSGSGTDFTLTISSLQPEDFATYYCQQSITLPPTFGCGTKVEIKGGGGSFWVLVVVGGVLACYSLLVTVAFIIFWVRSKRSRLLHSDYMNMTPRRPGPTRKHYQPYAPPRDFAAYRSRVKFSRSADAPAYQQGQNQLYNELNLGRREEYDVLDKRRGRDPEMGGKPRRKNPQEGLYNELQKDKMAEAYSEIGMKGERRRGKGHDGLYQGLSTATKDTYDALHMQALPPR

SEQ ID NO: 64 - protein, 125 aa, Artificial sequence
  Anti-DIG-ds VH
QVQLVESGGGLVKPGGSLRLSCAASGFTFSDYAMSWIRQAPGKCLEWVSSINIGATYIYYADSVKGRFTISRDNAKNSLYLQMNSLRAEDTAVYYCARPGSPYEYDKAYYSMAYWGQGTTVTVSS

SEQ ID NO: 65 - protein, 107 aa, Artificial sequence
  Anti-DIG-ds VL
DIQMTQSPSSLSASVGDRVTITCRASQDIKNYLNWYQQKPGKAPKLLIYYSSTLLSGVPSRFSGSGSGTDFTLTISSLQPEDFATYYCQQSITLPPTFGCGTKVEIK

SEQ ID NO: 66 - protein, 252 aa, Artificial sequence
  Anti-DIG-ds-scFv
QVQLVESGGGLVKPGGSLRLSCAASGFTFSDYAMSWIRQAPGKCLEWVSSINIGATYIYYADSVKGRFTISRDNAKNSLYLQMNSLRAEDTAVYYCARPGSPYEYDKAYYSMAYWGQGTTVTVSSGGGGSGGGGSGGGGSGGGGSDIQMTQSPSSLSASVGDRVTITCRASQDIKNYLNWYQQKPGKAPKLLIYYSSTLLSGVPSRFSGSGSGTDFTLTISSLQPEDFATYYCQQSITLPPTFGCGTKVEIK

SEQ ID NO: 67 - protein, 413 aa, Artificial sequence
  Anti-DIG-Fab-heavy chain-CD28ATD-CD28CSD-CD3zSSD fusion
QVQLVESGGGLVKPGGSLRLSCAASGFTFSDYAMSWIRQAPGKGLEWVSSINIGATYIYYADSVKGRFTISRDNAKNSLYLQMNSLRAEDTAVYYCARPGSPYEYDKAYYSMAYWGQGTTVTVSSASTKGPSVFPLAPSSKSTSGGTAALGCLVKDYFPEPVTVSWNSGALTSGVHTFPAVLQSSGLYSLSSVVTVPSSSLGTQTYICNVNHKPSNTKVDKKVEPKSCGGGGSFWVLVVVGGVLACYSLLVTVAFIIFWVRSKRSRLLHSDYMNMTPRRPGPTRKHYQPYAPPRDFAAYRSRVKFSRSADAPAYQQGQNQLYNELNLGRREEYDVLDKRRGRDPEMGGKPRRKNPQEGLYNELQKDKMAEAYSEIGMKGERRRGKGHDGLYQGLSTATKDTYDALHMQALPPR

SEQ ID NO: 68 - protein, 228 aa, Artificial sequence
  Anti-DIG-Fab heavy chain
QVQLVESGGGLVKPGGSLRLSCAASGFTFSDYAMSWIRQAPGKGLEWVSSINIGATYIYYADSVKGRFTISRDNAKNSLYLQMNSLRAEDTAVYYCARPGSPYEYDKAYYSMAYWGQGTTVTVSSASTKGPSVFPLAPSSKSTSGGTAALGCLVKDYFPEPVTVSWNSGALTSGVHTFPAVLQSSGLYSLSSVVTVPSSSLGTQTYICNVNHKPSNTKVDKKVEPKSC

SEQ ID NO: 69 - protein, 214 aa, Artificial sequence
  Anti-DIG-Fab light chain
DIQMTQSPSSLSASVGDRVTITCRASQDIKNYLNWYQQKPGKAPKLLIYYSSTLLSGVPSRFSGSGSGTDFTLTISSLQPEDFATYYCQQSITLPPTFGGGTKVEIKRTVAAPSVFIFPPSDEQLKSGTASVVCLLNNFYPREAKVQWKVDNALQSGNSQESVTEQDSKDSTYSLSSTLTLSKADYEKHKVYACEVTHQGLSSPVTKSFNRGEC

SEQ ID NO: 70 - protein, 125 aa, Artificial sequence
  Anti-DIG VH
QVQLVESGGGLVKPGGSLRLSCAASGFTFSDYAMSWIRQAPGKGLEWVSSINIGATYIYYADSVKGRFTISRDNAKNSLYLQMNSLRAEDTAVYYCARPGSPYEYDKAYYSMAYWGQGTTVTVSS

SEQ ID NO: 71 - protein, 107 aa, Artificial sequence
  Anti-DIG VL
DIQMTQSPSSLSASVGDRVTITCRASQDIKNYLNWYQQKPGKAPKLLIYYSSTLLSGVPSRFSGSGSGTDFTLTISSLQPEDFATYYCQQSITLPPTFGGGTKVEIK

SEQ ID NO: 72 - protein, 5 aa, Artificial sequence
  Anti-FITC CDR H1 Kabat
HYWMN

SEQ ID NO: 73 - protein, 19 aa, Artificial sequence
  Anti-FITC CDR H2 Kabat
QFRNKPYNYETYYSDSVKG

SEQ ID NO: 74 - protein, 7 aa, Artificial sequence
  Anti-FITC CDR H3 Kabat
ASYGMEY

SEQ ID NO: 75 - protein, 16 aa, Artificial sequence
  Anti-FITC CDR L1 Kabat
RSSQSLVHSNGNTYLR

SEQ ID NO: 76 - protein, 7 aa, Artificial sequence
  Anti-FITC CDR L2 Kabat
KVSNRVS

SEQ ID NO: 77 - protein, 9 aa, Artificial sequence
  Anti-FITC CDR L3 Kabat
SQSTHVPWT

SEQ ID NO: 78 - protein, 436 aa, Artificial sequence
  Anti-FITC-scFv-CD28ATD-CD28CSD-CD3zSSD fusion
GVKLDETGGGLVQPGGAMKLSCVTSGFTFGHYWMNWVRQSPEKGLEWVAQFRNKPYNYETYYSDSVKGRFTISRDDSKSSVYLQMNNLRVEDTGIYYCTGASYGMEYLGQGTSVTVSSGGGGSGGGGSGGGGSGGGGSDVVMTQTPLSLPVSLGDQASISCRSSQSLVHSNGNTYLRWYLQKPGQSPKVLIYKVSNRVSGVPDRFSGSGSGTDFTLKINRVEAEDLGVYFCSQSTHVPWTFGGGTKLEIKRGGGGSFWVLVVVGGVLACYSLLVTVAFIIFWVRSKRSRLLHSDYMNMTPRRPGPTRKHYQPYAPPRDFAAYRSRVKFSRSADAPAYQQGQNQLYNELNLGRREEYDVLDKRRGRDPEMGGKPRRKNPQEGLYNELQKDKMAEAYSEIGMKGERRRGKGHDGLYQGLSTATKDTYDALHMQALPPR

SEQ ID NO: 79 - protein, 250 aa, Artificial sequence
  Anti-FITC-scFv
GVKLDETGGGLVQPGGAMKLSCVTSGFTFGHYWMNWVRQSPEKGLEWVAQFRNKPYNYETYYSDSVKGRFTISRDDSKSSVYLQMNNLRVEDTGIYYCTGASYGMEYLGQGTSVTVSSGGGGSGGGGSGGGGSGGGGSDVVMTQTPLSLPVSLGDQASISCRSSQSLVHSNGNTYLRWYLQKPGQSPKVLIYKVSNRVSGVPDRFSGSGSGTDFTLKINRVEAEDLGVYFCSQSTHVPWTFGGGTKLEIK

SEQ ID NO: 80 - protein, 118 aa, Artificial sequence
  Anti-FITC VH
GVKLDETGGGLVQPGGAMKLSCVTSGFTFGHYWMNWVRQSPEKGLEWVAQFRNKPYNYETYYSDSVKGRFTISRDDSKSSVYLQMNNLRVEDTGIYYCTGASYGMEYLGQGTSVTVSS

SEQ ID NO: 81 - protein, 112 aa, Artificial sequence
  Anti-FITC VL
DVVMTQTPLSLPVSLGDQASISCRSSQSLVHSNGNTYLRWYLQKPGQSPKVLIYKVSNRVSGVPDRFSGSGSGTDFTLKINRVEAEDLGVYFCSQSTHVPWTFGGGTKLEIK

SEQ ID NO: 82 - protein, 5 aa, Artificial sequence
  Anti-HA CDR H1 Kabat
NYDMA

SEQ ID NO: 83 - protein, 17 aa, Artificial sequence
  Anti-HA CDR H2 Kabat
TISHDGRNTNYRDSVKG

SEQ ID NO: 84 - protein, 5 aa, Artificial sequence
  Anti-HA CDR H3 Kabat
PGFAH

SEQ ID NO: 85 - protein, 16 aa, Artificial sequence
  Anti-HA CDR L1 Kabat
RSSKTLLNTRGITSLY

SEQ ID NO: 86 - protein, 7 aa, Artificial sequence
  Anti-HA CDR L2 Kabat
RMSNLAS

SEQ ID NO: 87 - protein, 9 aa, Artificial sequence
  Anti-HA CDR L3 Kabat
AQFLEFPLT

SEQ ID NO: 88 - protein, 431 aa, Artificial sequence
  Anti-HA-scFv-CD28ATD-CD28CSD-CD3zSSD fusion
EVQLVESGGGLVQPGRSMKLSCAVSGFIFSNYDMAWVRQAPKKCLEWVATISHDGRNTNYRDSVKGRFTGSRDSAQSTLYLQMDSLRSEDTAIYFCAGPGFAHWGQGTLVTVSSGGGGSGGGGSGGGGSGGGGSDIVLTQAPLSVSVSPGESASISCRSSKTLLNTRGITSLYWYLQKPGKSPQLLIYRMSNLASGIPDRFSGSGSETHFTLQISKVETEDVGIYYCAQFLEFPLTFGCGTKLEIKGGGGSFWVLVVVGGVLACYSLLVTVAFIIFWVRSKRSRLLHSDYMNMTPRRPGPTRKHYQPYAPPRDFAAYRSRVKFSRSADAPAYQQGQNQLYNELNLGRREEYDVLDKRRGRDPEMGGKPRRKNPQEGLYNELQKDKMAEAYSEIGMKGERRRGKGHDGLYQGLSTATKDTYDALHMQALPPR

SEQ ID NO: 89 - protein, 246 aa, Artificial sequence
  Anti-HA-scFv
EVQLVESGGGLVQPGRSMKLSCAVSGFIFSNYDMAWVRQAPKKCLEWVATISHDGRNTNYRDSVKGRFTGSRDSAQSTLYLQMDSLRSEDTAIYFCAGPGFAHWGQGTLVTVSSGGGGSGGGGSGGGGSGGGGSDIVLTQAPLSVSVSPGESASISCRSSKTLLNTRGITSLYWYLQKPGKSPQLLIYRMSNLASGIPDRFSGSGSETHFTLQISKVETEDVGIYYCAQFLEFPLTFGCGTKLEIK

SEQ ID NO: 90 - protein, 114 aa, Artificial sequence
  Anti-HA VH
EVQLVESGGGLVQPGRSMKLSCAVSGFIFSNYDMAWVRQAPKKCLEWVATISHDGRNTNYRDSVKGRFTGSRDSAQSTLYLQMDSLRSEDTAIYFCAGPGFAHWGQGTLVTVSS

SEQ ID NO: 91 - protein, 112 aa, Artificial sequence
  Anti-HA VL
DIVLTQAPLSVSVSPGESASISCRSSKTLLNTRGITSLYWYLQKPGKSPQLLIYRMSNLASGIPDRFSGSGSETHFTLQISKVETEDVGIYYCAQFLEFPLTFGCGTKLEIK

SEQ ID NO: 92 - protein, 5 aa, Artificial sequence
  Anti-myc CDR H1 Kabat
HYGMS

SEQ ID NO: 93 - protein, 17 aa, Artificial sequence
  Anti-myc CDR H2 Kabat
TIGSRGTYTHYPDSVKG

SEQ ID NO: 94 - protein, 18 aa, Artificial sequence
  Anti-myc CDR H3 Kabat
RSEFYYYGNTYYYSAMDY

SEQ ID NO: 95 - protein, 15 aa, Artificial sequence
  Anti-myc CDR L1 Kabat
RASESVDNYGFSFMN

SEQ ID NO: 96 - protein, 7 aa, Artificial sequence
  Anti-myc CDR L2 Kabat
AISNRGS

SEQ ID NO: 97 - protein, 9 aa, Artificial sequence
  Anti-myc CDR L3 Kabat
QQTKEVPWT

SEQ ID NO: 98 - protein, 414 aa, Artificial sequence
  Anti-myc-Fab-heavy chain-CD28ATD-CD28CSD-CD3zSSD fusion
EVHLVESGGDLVKPGGSLKLSCAASGFTFSHYGMSWVRQTPDKRLEWVATIGSRGTYTHYPDSVKGRFTISRDNDKNALYLQMNSLKSEDTAMYYCARRSEFYYYGNTYYYSAMDYWGQGASVTVSSAKTTPPSVYPLAPGSAAQTNSMVTLGCLVKGYFPEPVTVTWNSGSLSSGVHTFPAVLQSDLYTLSSSVTVPSSTWPSETVTCNVAHPASSTKVDKKIVPRDCGGGGSFWVLVVVGGVLACYSLLVTVAFIIFWVRSKRSRLLHSDYMNMTPRRPGPTRKHYQPYAPPRDFAAYRSRVKFSRSADAPAYQQGQNQLYNELNLGRREEYDVLDKRRGRDPEMGGKPRRKNPQEGLYNELQKDKMAEAYSEIGMKGERRRGKGHDGLYQGLSTATKDTYDALHMQALPPR

SEQ ID NO: 99 - protein, 229 aa, Artificial sequence
  Anti-myc-Fab heavy chain
EVHLVESGGDLVKPGGSLKLSCAASGFTFSHYGMSWVRQTPDKRLEWVATIGSRGTYTHYPDSVKGRFTISRDNDKNALYLQMNSLKSEDTAMYYCARRSEFYYYGNTYYYSAMDYWGQGASVTVSSAKTTPPSVYPLAPGSAAQTNSMVTLGCLVKGYFPEPVTVTWNSGSLSSGVHTFPAVLQSDLYTLSSSVTVPSSTWPSETVTCNVAHPASSTKVDKKIVPRDC

SEQ ID NO: 100 - protein, 218 aa, Artificial sequence
  Anti-myc-Fab light chain
DIVLTQSPASLAVSLGQRATISCRASESVDNYGFSFMNWFQQKPGQPPKLLIYAISNRGSGVPARFSGSGSGTDFSLNIHPVEEDDPAMYFCQQTKEVPWTFGGGTKLEIKRADAAPTVSIFPPSSEQLTSGGASVVCFLNNFYPKDINVKWKIDGSERQNGVLNSWTDQDSKDSTYSMSSTLTLTKDEYERHNSYTCEATHKTSTSPIVKSFNRNEC

SEQ ID NO: 101 - protein, 127 aa, Artificial sequence
  Anti-myc VH
EVHLVESGGDLVKPGGSLKLSCAASGFTFSHYGMSWVRQTPDKRLEWVATIGSRGTYTHYPDSVKGRFTISRDNDKNALYLQMNSLKSEDTAMYYCARRSEFYYYGNTYYYSAMDYWGQGASVTVSS

SEQ ID NO: 102 - protein, 111 aa, Artificial sequence
  Anti-myc VL
DIVLTQSPASLAVSLGQRATISCRASESVDNYGFSFMNWFQQKPGQPPKLLIYAISNRGSGVPARFSGSGSGTDFSLNIHPVEEDDPAMYFCQQTKEVPWTFGGGTKLEIK

SEQ ID NO: 103 - protein, 9 aa, Artificial sequence
  HA tag
YPYDVPDYA

SEQ ID NO: 104 - protein, 10 aa, Artificial sequence
  Myc tag
EQKLISEEDL

SEQ ID NO: 105 - protein, 12 aa, Artificial sequence
  GCN4 tag
YHLENEVARLKK

SEQ ID NO: 106 - protein, 15 aa, Artificial sequence
  AviTag
GLNDIFEAQKIEWHE

SEQ ID NO: 107 - protein, 164 aa, Homo sapiens
MKWKALFTAAILQAQLPITEAQSFGLLDPKLCYLLDGILFIYGVILTALFLRVKFSRSADAPAYQQGQNQLYNELNLGRREEYDVLDKRRGRDPEMGGKPQRRKNPQEGLYNELQKDKMAEAYSEIGMKGERRRGKGHDGLYQGLSTATKDTYDALHMQALPPR

SEQ ID NO: 108 - DNA, 492 bp, Homo sapiens
atgaagtggaaggcgcttttcaccgcggccatcctgcaggcacagttgccgattacagaggcacagagctttggcctgctggatcccaaactctgctacctgctggatggaatcctcttcatctatggtgtcattctcactgccttgttcctgagagtgaagttcagcaggagcgcagagccccccgcgtaccagcagggccagaaccagctctataacgagctcaatctaggacgaagagaggagtacgatgttttggacaagagacgtggccgggaccctgagatggggggaaagccgagaaggaagaaccctcaggaaggcctgtacaatgaactgcagaaagataagatggcggaggcctacagtgagattgggatgaaaggcgagcgccggaggggcaaggggcacgatggcctttaccagggtctcagtacagccaccaaggacacctacgacgcccttcacatgcaggccctgccccctcgctaa

SEQ ID NO: 109 - protein, 164 aa, Mus musculus
MKWKVSVLACILHVRFPGAEAQSFGLLDPKLCYLLDGILFIYGVIITALYLRAKFSRSAETAANLQDPNQLYNELNLGRREEYDVLEKKRARDPEMGGKQQRRRNPQEGVYNALQKDKMAEAYSEIGTKGERRRGKGHDGLYQGLSTATKDTYDALHMQTLAPR

SEQ ID NO: 110 - DNA, 495 bp, Mus musculus
atgaagtggaaagtgtctgttctcgcctgcatcctccacgtgcggttcccaggagcagaggcacagagctttggtctgctggatcccaaactctgctacttgctagatggaatcctcttcatctacggagtcatcatcacagccctgtacctgagagcaaaattcagcaggagtgcagagactgctgccaacctgcaggaccccaaccagctctacaatgagctcaatctagggcgaagagaggaatatgacgtcttggagaagaagcgggctcgggatccagagatgggaggcaaacagcagaggaggaggaacccccaggaaggcgtatacaatgcactgcagaaagacaagatggcagaagcctacagtgagatcggcacaaaaggcgagaggcggagaggcaaggggcacgatggcctttaccagggtctcagcactgccaccaaggacacctatgatgccctgcatatgcagaccctggcccctcgctaa

SEQ ID NO: 111 - DNA, 660 bp, Homo sapiens
atgctgcgcctgctgctggcgctgaacctgtttccgagcattcaggtgaccggcaacaaaattctggtgaaacagagcccgatgctggtggcgtatgataacgcggtgaacctgagctgcaaatatagctataacctgtttagccgcgaatttcgcgcgagcctgcataaaggcctggatagcgcggtggaagtgtgcgtggtgtatggcaactatagccagcagctgcaggtgtatagcaaaaccggctttaactgcgatggcaaactgggcaacgaaagcgtgaccttttatctgcagaacctgtatgtgaaccagaccgatatttatttttgcaaaattgaagtgatgtatccgccgccgtatctggataacgaaaaaagcaacggcaccattattcatgtgaaaggcaaacatctgtgcccgagcccgctgtttccgggcccgagcaaaccgttttgggtgctggtggtggtgggcggcgtgctggcgtgctatagcctgctggtgaccgtggcgtttattattttttgggtgcgcagcaaacgcagccgcctgctgcatagcgattatatgaacatgaccccgcgccgcccgggcccgacccgcaaacattatcagccgtatgcgccgccgcgcgattttgcggcgtatcgcagc

SEQ ID NO: 112 - protein, 220 aa, Homo sapiens
MLRLLLALNLFPSIQVTGNKILVKQSPMLVAYDNAVNLSCKYSYNLFSREFRASLHKGLDSAVEVCVVYGNYSQQLQVYSKTGFNCDGKLGNESVTFYLQNLYVNQTDIYFCKIEVMYPPPYLDNEKSNGTIIHVKGKHLCPSPLFPGPSKPFWVLVVVGGVLACYSLLVTVAFIIFWVRSKRSRLLHSDYMNMTPRRPGPTRKHYQPYAPPRDFAAYRS

SEQ ID NO: 113 - DNA, 654 bp, Mus musculus
atgaccctgcgcctgctgtttctggcgctgaacttttttagcgtgcaggtgaccgaaaacaaaattctggtgaaacagagcccgctgctggtggtggatagcaacgaagtgagcctgagctgccgctatagctataacctgctggcgaaagaatttcgcgcgagcctgtataaaggcgtgaacagcgatgtggaagtgtgcgtgggcaacggcaactttacctatcagccgcagtttcgcagcaacgcggaatttaactgcgatggcgattttgataacgaaaccgtgacctttcgcctgtggaacctgcatgtgaaccataccgatatttatttttgcaaaattgaatttatgtatccgccgccgtatctggataacgaacgcagcaacggcaccattattcatattaaagaaaaacatctgtgccatacccagagcagcccgaaactgttttgggcgctggtggtggtggcgggcgtgctgttttgctatggcctgctggtgaccgtggcgctgtgcgtgatttggaccaacagccgccgcaaccgcctgctgcagagcgattatatgaacatgaccccgcgccgcccgggcctgacccgcaaaccgtatcagccgtatgcgccggcgcgcgattttgcggcgtatcgcccg

SEQ ID NO: 114 - protein, 218 aa, Mus musculus
MTLRLLFLALNFFSVQVTENKILVKQSPLLVVDSNEVSLSCRYSYNLLAKEFRASLYKGVNSDVEVCVGNGNFTYQPQFRSNAEFNCDGDFDNETVTFRLWNLHVNHTDIYFCKIEFMYPPPYLDNERSNGTIIHIKEKHLCHTQSSPKLFWALVVVAGVLFCYGLLVTVALCVIWTNSRRNRLLQSDYMNMTPRRPGLTRKPYQPYAPARDFAAYRP

SEQ ID NO: 115 - protein, 4 aa, Artificial sequence
  CD28 YMNM
YMNM

SEQ ID NO: 116 - protein, 4 aa, Artificial sequence
  CD28 PYAP
PYAP

SEQ ID NO: 117 - protein, 21 aa, Artificial sequence
  Signal peptide
ATMGWSCIILFLVATATGVHS

SEQ ID NO: 118 - DNA, 57 bp, Artificial sequence
  Signal peptide DNA sequence
atgggatggagctgtatcatcctcttcttggtagcaacagctaccggtgtgcactcc

SEQ ID NO: 119 - protein, 449 aa, Artificial sequence
  Anti-CD20 (GA101) PGLALA heavy chain
QVQLVQSGAEVKKPGSSVKVSCKASGYAFSYSWINWVRQAPGQGLEWMGRIFPGDGDTDYNGKFKGRVTITADKSTSTAYMELSSLRSEDTAVYYCARNVFDGYWLVYWGQGTLVTVSSASTKGPSVFPLAPSSKSTSGGTAALGCLVKDYFPEPVTVSWNSGALTSGVHTFPAVLQSSGLYSLSSVVTVPSSSLGTQTYICNVNHKPSNTKVDKKVEPKSCDKTHTCPPCPAPEAAGGPSVFLFPPKPKDTLMISRTPEVTCVVVDVSHEDPEVKFNWYVDGVEVHNAKTKPREEQYNSTYRVVSVLTVLHQDWLNGKEYKCKVSNKALGAPIEKTISKAKGQPREPQVYTLPPSRDELTKNQVSLTCLVKGFYPSDIAVEWESNGQPENNYKTTPPVLDSDGSFFLYSKLTVDKSRWQQGNVFSCSVMHEALHNHYTQKSLSLSPGK

SEQ ID NO: 120 - protein, 219 aa, Artificial sequence
  Anti-CD20 (GA101) light chain
DIVMTQTPLSLPVTPGEPASISCRSSKSLLHSNGITYLYWYLQKPGQSPQLLIYQMSNLVSGVPDRFSGSGSGTDFTLKISRVEAEDVGVYYCAQNLELPYTFGGGTKVEIKRTVAAPSVFIFPPSDEQLKSGTASVVCLLNNFYPREAKVQWKVDNALQSGNSQESVTEQDSKDSTYSLSSTLTLSKADYEKHKVYACEVTHQGLSSPVTKSFNRGEC

SEQ ID NO: 121 - protein, 451 aa, Artificial sequence
  Anti-CEA (CH1A1A98/992F1) PGLALA heavy chain
QVQLVQSGAEVKKPGASVKVSCKASGYTFTEFGMNWVRQAPGQGLEWMGWINTKTGEATYVEEFKGRVTFTTDTSTSTAYMELRSLRSDDTAVYYCARWDFAYYVEAMDYWGQGTTVTVSSASTKGPSVFPLAPSSKSTSGGTAALGCLVKDYFPEPVTVSWNSGALTSGVHTFPAVLQSSGLYSLSSVVTVPSSSLGTQTYICNVNHKPSNTKVDKKVEPKSCDKTHTCPPCPAPEAAGGPSVFLFPPKPKDTLMISRTPEVTCVVVDVSHEDPEVKFNWYVDGVEVHNAKTKPREEQYNSTYRVVSVLTVLHQDWLNGKEYKCKVSNKALGAPIEKTISKAKGQPREPQVCTLPPSRDELTKNQVSLSCAVKGFYPSDIAVEWESNGQPENNYKTTPPVLDSDGSFFLVSKLTVDKSRWQQGNVFSCSVMHEALHNHYTQKSLSLSPGK

SEQ ID NO: 122 - protein, 215 aa, Artificial sequence
  Anti-CEA (CH1A1A98/992F1) light chain
DIQMTQSPSSLSASVGDRVTITCKASAAVGTYVAWYQQKPGKAPKLLIYSASYRKRGVPSRFSGSGSGTDFTLTISSLQPEDFATYYCHQYYTYPLFTFGQGTKLEIKRTVAAPSVFIFPPSDEQLKSGTASVVCLLNNFYPREAKVQWKVDNALQSGNSQESVTEQDSKDSTYSLSSTLTLSKADYEKHKVYACEVTHQGLSSPVTKSFNRGEC

SEQ ID NO: 123 - protein, 330 aa, Artificial sequence [sequence omitted]

SEQ ID NO: 124 - protein, 372 aa, Artificial sequence
  Anti-WT1 (33F05) PGLALA heavy chain
QVQLQESGPGLVKPSETLSLTCTVSGGSINSYYWSWIRQPPGKGLEWIGYIYYSGSTNYNPSLKSRVTISVDTSKNQFSLKLSSVTAADTAVYYCARSYYEAFDYWGQGTLVTVSSSLGTQTYICNVNHKPSNTKVDKKVEPKSCDKTHTCPPCPAPEAAGGPSVFLFPPKPKDTLMISRTPEVTCVVVDVSHEDPEVKFNWYVDGVEVHNAKTKPREEQYNSTYRVVSVLTVLHQDWLNGKEYKCKVSNKALGAPIEKTISKAKGQPREPQVCTLPPSRDELTKNQVSLSCAVKGFYPSDIAVEWESNGQPENNYKTTPPVLDSDGSFFLVSKLTVDKSRWQQGNVFSCSVMHEALHNHYTQKSLSLSPGK

SEQ ID NO: 125 - protein, 214 aa, Artificial sequence
  Anti-WT1 (33F05) light chain
SSELTQDPAVSVALGQTVRITCQGDSLRSYYASWYQQKPGQAPVLVIYGKNNRPSGIPDRFSGSSSGNTASLTITGAQAEDEADYYCNSPDMNGNAVFGGGTKLTVLRTVAAPSVFIFPPSDEQLKSGTASVVCLLNNFYPREAKVQWKVDNALQSGNSQESVTEQDSKDSTYSLSSTLTLSKADYEKHKVYACEVTHQGLSSPVTKSFNRGEC

SEQ ID NO: 126 - protein, 376 aa, Artificial sequence
  Anti-WT1 (11D06) PGLALA heavy chain
QVQLVQSGAEVKKPGSSVKVSCKASGGTFSSYAISWVRQAPGQGLEWMGGIIPIFGTANYAQKFQGRVTITADKSTSTAYMELSSLRSEDTAVYYCARSIELWWGGFDYWGQGTTVTVSSSLGTQTYICNVNHKPSNTKVDKKVEPKSCDKTHTCPPCPAPEAAGGPSVFLFPPKPKDTLMISRTPEVTCVVVDVSHEDPEVKFNWYVDGVEVHNAKTKPREEQYNSTYRVVSVLTVLHQDWLNGKEYKCKVSNKALGAPIEKTISKAKGQPREPQVCTLPPSRDELTKNQVSLSCAVKGFYPSDIAVEWESNGQPENNYKTTPPVLDSDGSFFLVSKLTVDKSRWQQGNVFSCSVMHEALHNHYTQKSLSLSPGK

SEQ ID NO: 127 - protein, 213 aa, Artificial sequence
  Anti-WT1 (11D06) light chain
DIQMTQSPSTLSASVGDRVTITCRASQSISSWLAWYQQKPGKAPKLLIYDASSLESGVPSRFSGSGSGTEFTLTIGSLQPDDFATYYCQQYEDYTTFGQGTKVEIKRTVAAPSVFIFPPSDEQLKSGTASVVCLLNNFYPREAKVQWKVDNALQSGNSQESVTEQDSKDSTYSLSSTLTLSKADYEKHKVYACEVTHQGLSSPVTKSFNRGEC

SEQ ID NO: 128 - protein, 375 aa, Artificial sequence
  Anti-WT1 (33H09) PGLALA heavy chain
QVQLVQSGAEVKKPGSSVKVSCKASGGTFSSYAISWVRQAPGQGLEWMGGIIPIFGTANYAQKFQGRVTITADKSTSTAYMELSSLRSEDTAVYYCARGSYDLFSLDYWGQGTTVTVSSSLGTQTYICNVNHKPSNTKVDKKVEPKSCDKTHTCPPCPAPEAAGGPSVFLFPPKPKDTLMISRTPEVTCVVVDVSHEDPEVKFNWYVDGVEVHNAKTKPREEQYNSTYRVVSVLTVLHQDWLNGKEYKCKVSNKALGAPIEKTISKAKGQPREPQVCTLPPSRDELTKNQVSLSCAVKGFYPSDIAVEWESNGQPENNYKTTPPVLDSDGSFFLVSKLTVDKSRWQQGNVFSCSVMHEALHNHYTQKSLSLSPGK

SEQ ID NO: 129 - protein, 213 aa, Artificial sequence
  Anti-WT1 (33H09) light chain
DIQMTQSPSTLSASVGDRVTITCRASQSISSWLAWYQQKPGKAPKLLIYDASSLESGVPSRFSGSGSGTEFTLTISSLQPDDFATYYCQQYYDGITFGQGTKVEIKRTVAAPSVFIFPPSDEQLKSGTASVVCLLNNFYPREAKVQWKVDNALQSGNSQESVTEQDSKDSTYSLSSTLTLSKADYEKHKVYACEVTHQGLSSPVTKSFNRGEC

SEQ ID NO: 130 - protein, 375 aa, Artificial sequence
  Anti-WT1 (5E11) PGLALA heavy chain
QVQLVQSGAEVKKPGSSVKVSCKASGGTFSSYAISWVRQAPGQGLEWMGGIIPIFGTANYAQKFQGRVTITADKSTSTAYMELSSLRSEDTAVYYCARSSYDLYSFDYWGQGTTVTVSSSLGTQTYICNVNHKPSNTKVDKKVEPKSCDKTHTCPPCPAPEAAGGPSVFLFPPKPKDTLMISRTPEVTCVVVDVSHEDPEVKFNWYVDGVEVHNAKTKPREEQYNSTYRVVSVLTVLHQDWLNGKEYKCKVSNKALGAPIEKTISKAKGQPREPQVCTLPPSRDELTKNQVSLSCAVKGFYPSDIAVEWESNGQPENNYKTTPPVLDSDGSFFLVSKLTVDKSRWQQGNVFSCSVMHEALHNHYTQKSLSLSPGK

SEQ ID NO: 131 - protein, 215 aa, Artificial sequence
  Anti-WT1 (5E11) light chain
DIQMTQSPSTLSASVGDRVTITCRASQSISSWLAWYQQKPGKAPKLLIYDASSLESGVPSRFSGSGSGTEFTLTISSLQPDDFATYYCQQYSFPPMITFGQGTKVEIKRTVAAPSVFIFPPSDEQLKSGTASVVCLLNNFYPREAKVQWKVDNALQSGNSQESVTEQDSKDSTYSLSSTLTLSKADYEKHKVYACEVTHQGLSSPVTKSFNRGEC

SEQ ID NO: 132 - protein, 330 aa, Homo sapiens [sequence omitted]